European Patent Application EP 4 397 766 A1, published July 10, 2024. Title: ボルナウイルスベクターを利用した医薬組成物. Applicant: 国立大学法人京都大学. The sequence listing filed with the application follows.

SEQUENCE LISTING (13 sequences)

SEQ ID NO: 1 - protein, 10 aa, Mus musculus
GFSLNTSGMG

SEQ ID NO: 2 - protein, 7 aa, Mus musculus
IWWDDDK

SEQ ID NO: 3 - protein, 9 aa, Mus musculus
ARLGYAMDY

SEQ ID NO: 4 - protein, 7 aa, Mus musculus
QNVGGTN

SEQ ID NO: 5 - protein, 9 aa, Mus musculus
QQYYIYPYT

SEQ ID NO: 6 - protein, 154 aa, Homo sapiens [sequence omitted]

SEQ ID NO: 7 - DNA, 465 bp, Homo sapiens
  source 1..465: mol_type = other DNA
atggcgacgaaggccgtgtgcgtgctgaagggcgacggcccagtgcagggcatcatcaatttcgagcagaaggaaagtaatggaccagtgaaggtgtggggaagcattaaaggactgactgaaggcctgcatggattccatgttcatgagtttggagataatacagcaggctgtaccagtgcaggtcctcactttaatcctctatccagaaaacacggtgggccaaaggatgaagagaggcatgttggagacttgggcaatgtgactgctgacaaagatggtgtggccgatgtgtctattgaagattctgtgatctcactctcaggagaccattgcatcattggccgcacactggtggtccatgaaaaagcagatgacttgggcaaaggtggaaatgaagaaagtacaaagacaggaaacgctggaagtcgtttggcttgtggtgtaattgggatcgcccaataa

SEQ ID NO: 8 - protein, 116 aa, Mus musculus
QVTLKESGPGILQPSQTLSLTCSFSGFSLNTSGMGVGWIRQPSGRVLEWLAHIWWDDDKRYNPALKSRLTISKDTSTNQVFLKIASVDTTDTATYYCARLGYAMDYWGHGTSVTVS

SEQ ID NO: 9 - protein, 106 aa, Mus musculus
DIVMTQSQKFMSTSLGDRVSVTCKASQNVGTNVAWYQQKPGQSPKALIYSASYRYSGVPDRFTGSGSGTDFTLTISNVQSEDLAEYFCQQYYIYPYTFGGGTKLEI

SEQ ID NO: 10 - DNA, 348 bp, Mus musculus
  source 1..348: mol_type = other DNA
caggttactctgaaagagtctggccctgggatattgcagccctcccagaccctcagtctgacttgttctttctctgggttttcactgaacacttctggtatgggtgtaggctggattcgtcagccttcagggagggttctggagtggctggcacacatttggtgggatgatgacaagcgctataacccagccctgaagagccgactgacaatctccaaggatacctccaccaaccaggtattcctcaagatcgccagtgtggacactacagatactgccacatactactgtgctcgacttggctatgctatggactactggggtcacggaacctcagtcaccgtctcc

SEQ ID NO: 11 - DNA, 318 bp, Mus musculus
  source 1..318: mol_type = other DNA
gacattgtgatgacccagtctcaaaaattcatgtccacatcactaggagacagggtcagcgtcacctgcaaggccagtcagaatgtgggtactaatgtagcctggtatcaacagaaaccagggcaatctcctaaagcactgatttactcggcatcctaccggtacagtggagtccctgatcgcttcacaggcagtggatctgggacagatttcactctcaccatcagcaatgtgcagtctgaagacttggcagagtatttctgtcagcaatattacatctatccgtacacgttcggaggggggaccaagctggaaata

SEQ ID NO: 12 - DNA, 348 bp, synthetic construct
  source 1..348: mol_type = other DNA
caggttactctgaaggagtctggccctgggatactgcagccctcacagaccctgagtctgacttgttccttctctggattttcactgaacacctctggtatgggtgtaggctggattcgtcagccttccgggagggttctggagtggctggctcacatctggtgggatgatgataagcgctataaccctgccctgaagagccgactgaccatctctaaggatacctccaccaaccaggtattcctcaagatcgccagtgtggacaccaccgatactgctacatactactgtgctcgtcttggctatgctatggactactggggtcacggaacctcagtcaccgtctcc

SEQ ID NO: 13 - DNA, 318 bp, synthetic construct
  source 1..318: mol_type = other DNA
gacattgtgatgacccagtctcaaaaattcatgtccacctcacttggagaccgagtctcagtcacctgcaaggcttcccagaatgtgggtacaaatgtagcctggtatcagcagaaaccaggacagtctcctaaggcactgatttactcggcttcctaccgttactccggagtccctgatcgtttcacaggtagtggatctggaacagatttcaccctgaccatcagcaatgttcagtctgaagatttggcagagtatttctgccagcaatattacatctatccgtacacgttcggaggaggaaccaagctggaaatt